European Patent Application EP 4 206 316 A1, published July 5, 2023. Title: Lactobacillus plantarum microorganism with anticancer activity, composition comprising the same and method for preventing or treating cancer. Applicant: Medytox Inc. The sequence listing filed with the application follows.

SEQUENCE LISTING (3 sequences)

SEQ ID NO: 1 - DNA, 20 bp, Artificial
  primer
agagtttgatcmtggctcag

SEQ ID NO: 2 - DNA, 22 bp, Artificial
  Primer
tacggytaccttgttacgactt

SEQ ID NO: 3 - DNA, 1356 bp, Lactobacillus plantarum LMT17-31
tgcttgcatcatgatttacatttgagtgagtggcgaactggtgagtaacacgtgggaaacctgcccagaagcgggggataacacctggaaacagatgctaataccgcataacaacttggaccgcatggtccgagcttgaaagatggcttcggctatcacttttggatggtcccgcggcgtattagctagatggtggggtaacggctcaccatggcaatgatacgtagccgacctgagagggtaatcggccacattgggactgagacacggcccaaactcctacgggaggcagcagtagggaatcttccacaatggacgaaagtctgatggagcaacgccgcgtgagtgaagaagggtttcggctcgtaaaactctgttgttaaagaagaacatatctgagagtaactgttcaggtattgacggtatttaaccagaaagccacggctaactacgtgccagcagccgcggtaatacgtaggtggcaagcgttgtccggatttattgggcgtaaagcgagcgcaggcggttttttaagtctgatgtgaaagccttcggctcaaccgaagaagtgcatcggaaactgggaaacttgagtgcagaagaggacagtggaactccatgtgtagcggtgaaatgcgtagatatatggaagaacaccagtggcgaaggcggctgtctggtctgtaactgacgctgaggctcgaaagtatgggtagcaaacaggattagataccctggtagtccataccgtaaacgatgaatgctaagtgttggagggtttccgcccttcagtgctgcagctaacgcattaagcattccgcctggggagtacggccgcaaggctgaaactcaaaggaattgacgggggcccgcacaagcggtggagcatgtggtttaattcgaagctacgcgaagaaccttaccaggtcttgacatactatgcaaatctaagagattagacgttcccttcggggacatggatacaggtggtgcatggttgtcgtcagctcgtgtcgtgagatgttgggttaagtcccgcaacgagcgcaacccttattatcagttgccagcattaagttgggcactctggtgagactgccggtgacaaaccggaggaaggtggggatgacgtcaaatcatcatgccccttatgacctgggctacacacgtgctacaatggatggtacaacgagttgcgaactcgcgagagtaagctaatctcttaaagccattctcagttcggattgtaggctgcaactcgcctacatgaagtcggaatcgctagtaatcgcggatcagcatgccgcggtgaatacgttcccgggccttgtacacaccgcccgtcacaccatgaga